European Patent Application EP 4 574 983 A1, published June 25, 2025. Title: Verfahren zur Herstellung von Allitol. Applicant: Annikki GmbH. Application EP. The sequence listing filed with the application follows.

SEQUENCE LISTING (6 sequences)

SEQ ID NO: 1 - DNA, 785 bp, Gluconobacter frateurii
  source 1..785: mol_type = genomic DNA
atgacacagtctcttcagggcaagatcgtcgccattactggcgcggcttcgggcattggcctcgaatgcgcccgctatctcatcgaagctggcgcggtggtctatcttctggaccgtgacgccaaaactctcgaagacaaaacggcagaactcggcagccaggcccatgcgatcatcgtcgatctcttcgactacaaaaccgtagatgctgcggtcgcgcagatcgttgaggagcagggccggatcgatgttttccacgccaacgccggcgcgtatgtgggcggcaatgtctgggaaggggatcccgatagctgggatgcgatgctgcacctgaacatcaatgcagctttccgctcggtccgtgccgtgctgccgcagatgatgaagcaggaaagtggcgatatcgtcatgaccagctcgatcgcgggcatgatccccatcatggccgagccgatctacacggcctcgaaacatgccgtgcaggcattcgtacatacggtgcgccgacaggtcgcgaagtatggaattcgtgtgggtgcaatccagcctggtcctgtagtcacgcctttgctgaaagactgggatcaggcccgtcttgaagccaacatcaaagcgggtgccctgatggaagccaaggaagtcgccgaagccctgatcttcatcctgacacgttcaaagggtgtcatggtgcgggatctggtcgttctgccacataacttcgacgcctaagcttaagcggccgcactcgagcaccaccaccaccaccactgagatccggctgctaa

SEQ ID NO: 2 - protein, 242 aa, Gluconobacter frateurii
MTQSLQGKIVAITGAASGIGLECARYLIEAGAVVYLLDRDAKTLEDKTAELGSQAHAIIVDLFDYKTVDAAVAQIVEEQGRIDVFHANAGAYVGGNVWEGDPDSWDAMLHLNINAAFRSVRAVLPQMMKQESGDIVMTSSIAGMIPIMAEPIYTASKHAVQAFVHTVRRQVAKYGIRVGAIQPGPVVTPLLKDWDQARLEANIKAGALMEAKEVAEALIFILTRSKGVMVRDLVVLPHNFDA

SEQ ID NO: 3 - DNA, 1014 bp, Geobacillus stearothermophilus
  source 1..1014: mol_type = genomic DNA
atgaaagctgcagttgtggaacaatttaaaaagccgttacaagtgaaagaagtggaaaaacctaagatctcatacggggaagtattagtgcgcatcaaagcgtgtggggtatgccatacagacttgcatgccgcacatggcgactggcctgtaaagcctaaactgcctctcattcctggccatgaaggcgtcggtgtaattgaagaagtaggtcctggggtaacacatttaaaagttggagatcgcgtaggtatcccttggctttattcggcgtgcggtcattgtgactattgcttaagcggacaagaaacattatgcgaacgtcaacaaaacgctggctattccgtcgatggtggttatgctgaatattgccgtgctgcagccgattatgtcgtaaaaattcctgataacttatcgtttgaagaagccgctccaatcttttgcgctggtgtaacaacatataaagcgctcaaagtaacaggcgcaaaaccaggtgaatgggtagccatttacggtatcggcgggcttggacatgtcgcagtccaatacgcaaaggcgatggggttaaacgtcgttgctgtcgatttaggtgatgaaaaacttgagcttgctaaacaacttggtgcagatcttgtcgtcaatccgaaacatgatgatgcagcacaatggataaaagaaaaagtgggcggtgtgcatgcgactgtcgtcacagctgtttcaaaagccgcgttcgaatcagcctacaaatccattcgtcgcggtggtgcttgcgtactcgtcggattaccgccggaagaaatacctattccaattttcgatacagtattaaatggagtaaaaattattggttctatcgttggtacgcgcaaagacttacaagaggcacttcaatttgcagcagaaggaaaagtaaaaacaattgtcgaagtgcaaccgcttgaaaacattaacgacgtattcgatcgtatgttaaaagggcaaattaacggccgcgtcgtgttaaaagtagattaa

SEQ ID NO: 4 - protein, 337 aa, Geobacillus stearothermophilus
MKAAVVEQFKKPLQVKEVEKPKISYGEVLVRIKACGVCHTDLHAAHGDWPVKPKLPLIPGHEGVGVIEEVGPGVTHLKVGDRVGIPWLYSACGHCDYCLSGQETLCERQQNAGYSVDGGYAEYCRAAADYVVKIPDNLSFEEAAPIFCAGVTTYKALKVTGAKPGEWVAIYGIGGLGHVAVQYAKAMGLNVVAVDLGDEKLELAKQLGADLVVNPKHDDAAQWIKEKVGGVHATVVTAVSKAAFESAYKSIRRGGACVLVGLPPEEIPIPIFDTVLNGVKIIGSIVGTRKDLQEALQFAAEGKVKTIVEVQPLENINDVFDRMLKGQINGRVVLKVD

SEQ ID NO: 5 - DNA, 786 bp, Priestia megaterium
  source 1..786: mol_type = genomic DNA
atgtatacagatttaaaagataaagtagttgtaattacaggtggatcaacaggtttaggacgcgcaatggctgttcgtttcggtcaagaagaagcaaaagttgttattaactattacaacaatgaagaagaagctttagatgcgaaaaaagaagtagaagaagcaggcggacaagcaatcatcgttcaaggcgacgtaacaaaagaagaagatgttgtaaaccttgttcaaacagctattaaagaattcggtacattagacgttatgattaataacgctggtgttgaaaacccagttccttctcatgagttatctttagacaactggaataaagttattgatacaaacttaacaggtgcattcttaggaagccgtgaagcaatcaaatattttgttgaaaacgacattaaaggaaacgttattaacatgtctagtgttcatgaaatgattccttggccattatttgttcattacgcagcaagtaaaggcggtatgaaactaatgacggaaacattggctcttgaatatgcgccaaaaggtatccgcgtaaataacattggaccaggtgcgatgaacacaccaattaacgcagagaaatttgcagatcctgtacaacgtgcagacgtagaaagcatgattccaatgggttacatcggtaaaccagaagaagtagcagcagttgcagcattcttagcatcatcacaagcaagctatgtaacaggtattacattatttgctgatggtggtatgacgaaatacccttctttccaagcaggaagaggctaa

SEQ ID NO: 6 - protein, 261 aa, Priestia megaterium
MYTDLKDKVVVITGGSTGLGRAMAVRFGQEEAKVVINYYNNEEEALDAKKEVEEAGGQAIIVQGDVTKEEDVVNLVQTAIKEFGTLDVMINNAGVENPVPSHELSLDNWNKVIDTNLTGAFLGSREAIKYFVENDIKGNVINMSSVHEMIPWPLFVHYAASKGGMKLMTETLALEYAPKGIRVNNIGPGAMNTPINAEKFADPVQRADVESMIPMGYIGKPEEVAAVAAFLASSQASYVTGITLFADGGMTKYPSFQAGRG